European Patent Application EP 4 512 243 A1, published February 26, 2025. Title: BINDING MOLECULES. Applicant: Kymab Limited. Application GB. The sequence listing filed with the application follows.

SEQUENCE LISTING (19 sequences)

SEQ ID NO: 1 - RNA, 20 nt, synthetic construct
  source 1..20: mol_type = other RNA
gatgccactggggacgccaa

SEQ ID NO: 2 - RNA, 20 nt, synthetic construct
  source 1..20: mol_type = other RNA
aagtcccttggcgtccccag

SEQ ID NO: 3 - RNA, 20 nt, synthetic construct
  source 1..20: mol_type = other RNA
ggagccggctgagagaagtt

SEQ ID NO: 4 - RNA, 20 nt, synthetic construct
  source 1..20: mol_type = other RNA
gtggagataatctgtcctaa

SEQ ID NO: 5 - RNA, 20 nt, synthetic construct
  source 1..20: mol_type = other RNA
tcactacttgcgtcccgctg

SEQ ID NO: 6 - RNA, 20 nt, synthetic construct
  source 1..20: mol_type = other RNA
gcccagccaccgggacagag

SEQ ID NO: 7 - DNA, 111 bp, Homo sapiens
  source 1..111: mol_type = genomic DNA
cctgaggcctcaccacggccccgccacccctgatagccatgacagtctctctagagagggaagagagggagccgaagggggcgggagtggcgggcaccgggctgacacgtg

SEQ ID NO: 8 - RNA, 20 nt, synthetic construct
  source 1..20: mol_type = other RNA
gattgggagttactggaatc

SEQ ID NO: 9 - RNA, 20 nt, synthetic construct
  source 1..20: mol_type = other RNA
gcccccagaggtgctcttgg

SEQ ID NO: 10 - DNA, 120 bp, synthetic construct
  source 1..120: mol_type = other DNA
ctgcgccctgggcccagctctgtcccacaccgcggtcacatggcaccacctctcttgcagagcccaaatcttgtgacaaaactcacacatgcccaccgtgcccaggtaagccagcccagg

SEQ ID NO: 11 - DNA, 75 bp, Homo sapiens
  source 1..75: mol_type = genomic DNA
cctccaccaagggcccatcggtcttccccctggcaccctcctccaatccagtaactcccaatcttctctctgcag

SEQ ID NO: 12 - DNA, 72 bp, Homo sapiens
  source 1..72: mol_type = genomic DNA
cctccaccaagggcccatcggtcttccccctggcaccctcctccactgcagagagaagattgggagttactg

SEQ ID NO: 13 - RNA, 20 nt, synthetic construct
  source 1..20: mol_type = other RNA
tgggttcttaactgtccgcg

SEQ ID NO: 14 - RNA, 20 nt, synthetic construct
  source 1..20: mol_type = other RNA
cacacatgcccaccgtgccc

SEQ ID NO: 15 - DNA, 234 bp, synthetic construct
  source 1..234: mol_type = other DNA
ccagccaggcgcacacccaatgcccgtgagcccagacactggacgctgaacgtcgcggacagttaagaacccacgggcctctgcgccctgggcccagctctgtcccacaccgcggtcacatggcaccacctctcttgcagagcctaaatcttgtgacaaaactcacacctgtcctccgtgcccaggtaagccagcccaggcctcgccctccagctcaaggcgggacaggtgccc

SEQ ID NO: 16 - DNA, 250 bp, Homo sapiens
  source 1..250: mol_type = genomic DNA
gtccctgaggtggcaccgatggccagagctgaggccaagctagaggccctggactgtgctgactcccggcagacacagagcgctgacctggctgccgagccccgcccccgctgaacgtcgcggacagttaagaacccacgggcctctgcgccctgggcccagctctgtcccacaccgcggtcacatggcaccacctctcttgcagagcctaaatcttgtgacaaaactcacacctgtcctccgtgcccag

SEQ ID NO: 17 - DNA, 157 bp, Homo sapiens
  source 1..157: mol_type = genomic DNA
agcccagacactggacgctgaacgtcgcggacagttaagaacccacgggcctctgcgccctgggcccagctctgtcccacaccgcggtcacatggcaccacctctcttgcagagcctaaatcttgtgacaaaacttacacctgtcctccgtgcccag

SEQ ID NO: 18 - protein, 15 aa, Homo sapiens
EPKSCDKTYTCPPCP

SEQ ID NO: 19 - DNA, 210 bp, Homo sapiens
  source 1..210: mol_type = genomic DNA
ccagccaggcgcacacccaatgcccgtgagcccagacactggacgctgaacctcgcccagacactggacgctgaacgtcgcggacagttaagaacccacgggcctctgcgccctgggcccagctctgtcccacaccgcggtcacatggcaccacctctcttgcagagcctaaatcttgtgacaaaactcacacctgtcctccgtgcccag